European Patent Application EP 4 299 597 A1, published January 3, 2024. Title: Dual-target STAR targeting CD19 and CD22. Applicant: CHINA IMMUNOTECH (BEIJING) BIOTECHNOLOGY CO., LTD. The sequence listing filed with the application follows.

SEQUENCE LISTING (84 sequences)

SEQ ID NO: 1 - protein, 141 aa, Homo sapiens
DIQNPDPAVYQLRDSKSSDKSVCLFTDFDSQTNVSQSKDSDVYITDKTVLDMRSMDFKSNSAVAWSNKSDFACANAFNNSIIPEDTFFPSPESSCDVKLVEKSFETDTNLNFQNLSVIGFRILLLKVAGFNLLMTLRLWSS

SEQ ID NO: 2 - protein, 137 aa, Mus musculus
DIQNPEPAVYQLKDPRSQDSTLCLFTDFDSQINVPKTMESGTFITDKTVLDMKAMDSKSNGAIAWSNQTSFTCQDIFKETNATYPSSDVPCDATLTEKSFETDMNLNFQNLSVMGLRILLLKVAGFNLLMTLRLWSS

SEQ ID NO: 3 - protein, 137 aa, Artificial sequence
  mouse T cell receptor alpha chain constant region containing cysteine substitution and modification of hydrophobic region
DIQNPEPAVYQLKDPRSQDSTLCLFTDFDSQINVPKTMESGTFITDKCVLDMKAMDSKSNGAIAWSNQTSFTCQDIFKETNATYPSSDVPCDATLTEKSFETDMNLNFQNLLVIVLRILLLKVAGFNLLMTLRLWSS

SEQ ID NO: 4 - protein, 133 aa, artificial sequence
  mouse T cell receptor alpha chain constant region containing N-terminal modification, cysteine substitution and modification of transmembrane hydrophobic region
DIQNPDPAVYQLRDDSTLCLFTDFDSQINVPKTMESGTFITDKCVLDMKAMDSKSNGAIAWSNQTSFTCQDIFKETNATYPSSDVPCDATLTEKSFETDMNLNFQNLLVIVLRILLLKVAGFNLLMTLRLWSS

SEQ ID NO: 5 - protein, 176 aa, Homo sapiens
DLKNVFPPEVAVFEPSEAEISHTQKATLVCLATGFYPDHVELSWWVNGKEVHSGVSTDPQPLKEQPALNDSRYCLSSRLRVSATFWQNPRNHFRCQVQFYGLSENDEWTQDRAKPVTQIVSAEAWGRADCGFTSESYQQGVLSATILYEILLGKATLYAVLVSALVLMAMVKRKDF

SEQ ID NO: 6 - protein, 172 aa, Mus musculus
DLRNVTPPKVSLFEPSKAEIANKQKATLVCLARGFFPDHVELSWWVNGKEVHSGVSTDPQAYKESNYSYCLSSRLRVSATFWHNPRNHFRCQVQFHGLSEEDKWPEGSPKPVTQNISAEAWGRADCGITSASYQQGVLSATILYEILLGKATLYAVLVSTLVVMAMVKRKNS

SEQ ID NO: 7 - protein, 172 aa, Artificial sequence
  mouse T cell receptor beta chain constant region containing cysteine substitution
DLRNVTPPKVSLFEPSKAEIANKQKATLVCLARGFFPDHVELSWWVNGKEVHSGVCTDPQAYKESNYSYCLSSRLRVSATFWHNPRNHFRCQVQFHGLSEEDKWPEGSPKPVTQNISAEAWGRADCGITSASYQQGVLSATILYEILLGKATLYAVLVSTLVVMAMVKRKNS

SEQ ID NO: 8 - protein, 166 aa, Artificial sequence
  mouse T cell receptor beta chain constant region containing N-terminal modification, and cysteine substitution
DLKNVFPPEVAVFEPSAEIATLVCLARGFFPDHVELSWWVNGKEVHSGVCTDPQAYKESNYSYCLSSRLRVSATFWHNPRNHFRCQVQFHGLSEEDKWPEGSPKPVTQNISAEAWGRADCGITSASYQQGVLSATILYEILLGKATLYAVLVSTLVVMAMVKRKNS

SEQ ID NO: 9 - protein, 120 aa, Artificial sequence
  Anti-CD19 FMC63 VH
EVKLQESGPGLVAPSQSLSVTCTVSGVSLPDYGVSWIRQPPRKGLEWLGVIWGSETTYYNSALKSRLTIIKDNSKSQVFLKMNSLQTDDTAIYYCAKHYYYGGSYAMDYWGQGTSVTVSS

SEQ ID NO: 10 - protein, 107 aa, Artificial sequence
  Anti-CD19 FMC63 VL
DIQMTQTTSSLSASLGDRVTISCRASQDISKYLNWYQQKPDGTVKLLIYHTSRLHSGVPSRFSGSGSGTDYSLTISNLEQEDIATYFCQQGNTLPYTFGGGTKLEIT

SEQ ID NO: 11 - protein, 124 aa, Artificial sequence
  Anti-CD22 M971 VH
QVQLQQSGPGLVKPSQTLSLTCAISGDSVSSNSAAWNWIRQSPSRGLEWLGRTYYRSKWYNDYAVSVKSRITINPDTSKNQFSLQLNSVTPEDTAVYYCAREVTGDLEDAFDIWGQGTMVTVSS

SEQ ID NO: 12 - protein, 107 aa, Artificial sequence
  Anti-CD22 M971 VL
DIQMTQSPSSLSASVGDRVTITCRASQTIWSYLNWYQQRPGKAPNLLIYAASSLQSGVPSRFSGRGSGTDFTLTISSLQAEDFATYYCQQSYSIPQTFGQGTKLEIK

SEQ ID NO: 13 - protein, 57 aa, Artificial sequence
  CD8 hinge region amino acid sequence
SHFVPVFLPAKPTTTPAPRPPTPAPTIASQPLSLRPEACRPAAGGAVHTRGLDFACD

SEQ ID NO: 14 - protein, 37 aa, Artificial sequence
  OX40 endodomain
RRDQRLPPDAHKPPGGGSFRTPIQEEQADAHSTLAKI

SEQ ID NO: 15 - protein, 15 aa, Artificial sequence
  (G4S)3 linker
GGGGSGGGGSGGGGS

SEQ ID NO: 16 - protein, 379 aa, Artificial sequence
  CD19-22 STAR(CT) alpha chain
DIQMTQTTSSLSASLGDRVTISCRASQDISKYLNWYQQKPDGTVKLLIYHTSRLHSGVPSRFSGSGSGTDYSLTISNLEQEDIATYFCQQGNTLPYTFGGGTKLEITGGGGSGGGGSGGGGSEVKLQESGPGLVAPSQSLSVTCTVSGVSLPDYGVSWIRQPPRKGLEWLGVIWGSETTYYNSALKSRLTIIKDNSKSQVFLKMNSLQTDDTAIYYCAKHYYYGGSYAMDYWGQGTSVTVSSDIQNPEPAVYQLKDPRSQDSTLCLFTDFDSQINVPKTMESGTFITDKCVLDMKAMDSKSNGAIAWSNQTSFTCQDIFKETNATYPSSDVPCDATLTEKSFETDMNLNFQNLLVIVLRILLLKVAGFNLLMTLRLWSS

SEQ ID NO: 17 - protein, 478 aa, Artificial sequence
  CD19-22 STAR(CT) beta chain
DIQMTQSPSSLSASVGDRVTITCRASQTIWSYLNWYQQRPGKAPNLLIYAASSLQSGVPSRFSGRGSGTDFTLTISSLQAEDFATYYCQQSYSIPQTFGQGTKLEIKGGGGSGGGGSGGGGSQVQLQQSGPGLVKPSQTLSLTCAISGDSVSSNSAAWNWIRQSPSRGLEWLGRTYYRSKWYNDYAVSVKSRITINPDTSKNQFSLQLNSVTPEDTAVYYCAREVTGDLEDAFDIWGQGTMVTVSSEFSHFVPVFLPAKPTTTPAPRPPTPAPTIASQPLSLRPEACRPAAGGAVHTRGLDFACDEDLRNVTPPKVSLFEPSKAEIANKQKATLVCLARGFFPDHVELSWWVNGKEVHSGVCTDPQAYKESNYSYCLSSRLRVSATFWHNPRNHFRCQVQFHGLSEEDKWPEGSPKPVTQNISAEAWGRADCGITSASYQQGVLSATILYEILLGKATLYAVLVSTLVVMAMVKRKNS

SEQ ID NO: 18 - protein, 429 aa, Artificial sequence
  CD19-22 STAR-OX40 alpha chain(CT)
DIQMTQTTSSLSASLGDRVTISCRASQDISKYLNWYQQKPDGTVKLLIYHTSRLHSGVPSRFSGSGSGTDYSLTISNLEQEDIATYFCQQGNTLPYTFGGGTKLEITGGGGSGGGGSGGGGSEVKLQESGPGLVAPSQSLSVTCTVSGVSLPDYGVSWIRQPPRKGLEWLGVIWGSETTYYNSALKSRLTIIKDNSKSQVFLKMNSLQTDDTAIYYCAKHYYYGGSYAMDYWGQGTSVTVSSDIQNPEPAVYQLKDPRSQDSTLCLFTDFDSQINVPKTMESGTFITDKCVLDMKAMDSKSNGAIAWSNQTSFTCQDIFKETNATYPSSDVPCDATLTEKSFETDMNLNFQNLLVIVLRILLLKVAGFNLLMTLRLWGGGGSGGGGSGGGGSRRDQRLPPDAHKPPGGGSFRTPIQEEQADAHSTLAKI

SEQ ID NO: 19 - protein, 478 aa, Artificial sequence; identical to SEQ ID NO: 17
  CD19-22 STAR-OX40 beta chain(CT)

SEQ ID NO: 20 - protein, 415 aa, Artificial sequence
  CD19-STAR(CT) beta chain
DIQMTQTTSSLSASLGDRVTISCRASQDISKYLNWYQQKPDGTVKLLIYHTSRLHSGVPSRFSGSGSGTDYSLTISNLEQEDIATYFCQQGNTLPYTFGGGTKLEITGGGGSGGGGSGGGGSEVKLQESGPGLVAPSQSLSVTCTVSGVSLPDYGVSWIRQPPRKGLEWLGVIWGSETTYYNSALKSRLTIIKDNSKSQVFLKMNSLQTDDTAIYYCAKHYYYGGSYAMDYWGQGTSVTVSSEDLRNVTPPKVSLFEPSKAEIANKQKATLVCLARGFFPDHVELSWWVNGKEVHSGVCTDPQAYKESNYSYCLSSRLRVSATFWHNPRNHFRCQVQFHGLSEEDKWPEGSPKPVTQNISAEAWGRADCGITSASYQQGVLSATILYEILLGKATLYAVLVSTLVVMAMVKRKNS

SEQ ID NO: 21 - protein, 137 aa, Artificial sequence; identical to SEQ ID NO: 3
  alpha chain of CD19-STAR(CT ) or CD22-STAR(CT)

SEQ ID NO: 22 - protein, 478 aa, Artificial sequence; identical to SEQ ID NO: 17
  beta chain of CD22-STAR(CT) or M971(CD8h)ba

SEQ ID NO: 23 - protein, 137 aa, Artificial sequence; identical to SEQ ID NO: 3
  CD22-STAR(CT) alpha chain

SEQ ID NO: 24 - protein, 711 aa, Artificial sequence
  CD19-22 CAR
DIQMTQTTSSLSASLGDRVTISCRASQDISKYLNWYQQKPDGTVKLLIYHTSRLHSGVPSRFSGSGSGTDYSLTISNLEQEDIATYFCQQGNTLPYTFGGGTKLEITGGGGSQVQLQQSGPGLVKPSQTLSLTCAISGDSVSSNSAAWNWIRQSPSRGLEWLGRTYYRSKWYNDYAVSVKSRITINPDTSKNQFSLQLNSVTPEDTAVYYCAREVTGDLEDAFDIWGQGTMVTVSSGSTSGSGKPGSGEGSTKGDIQMTQSPSSLSASVGDRVTITCRASQTIWSYLNWYQQRPGKAPNLLIYAASSLQSGVPSRFSGRGSGTDFTLTISSLQAEDFATYYCQQSYSIPQTFGQGTKLEIKGGGGSEVKLQESGPGLVAPSQSLSVTCTVSGVSLPDYGVSWIRQPPRKGLEWLGVIWGSETTYYNSALKSRLTIIKDNSKSQVFLKMNSLQTDDTAIYYCAKHYYYGGSYAMDYWGQGTSVTVSSSGTTTPAPRPPTPAPTIASQPLSLRPEACRPAAGGAVHTRGLDFACDIYIWAPLAGTCGVLLLSLVITLYCKRGRKKLLYIFKQPFMRPVQTTQEEDGCSCRFPEEEEGGCELRVKFSRSADAPAYQQGQNQLYNELNLGRREEYDVLDKRRGRDPEMGGKPRRKNPQEGLYNELQKDKMAEAYSEIGMKGERRRGKGHDGLYQGLSTATKDTYDALHMQALPPR

SEQ ID NO: 25 - protein, 8 aa, Artificial sequence
  FMC63 heavy chain variable region CDR1 amino acid sequence
GVSLPDYG

SEQ ID NO: 26 - protein, 7 aa, Artificial sequence
  FMC63 heavy chain variable region CDR2 amino acid sequence
IWGSETT

SEQ ID NO: 27 - protein, 2 aa, Artificial sequence
  FMC63 heavy chain variable region CDR3 amino acid sequence
AK

SEQ ID NO: 28 - protein, 6 aa, Artificial sequence
  FMC63 light chain variable region CDR1 amino acid sequence
QDISKY

SEQ ID NO: 29 - protein, 3 aa, Artificial sequence
  FMC63 light chain variable region CDR2 amino acid sequence
HTS

SEQ ID NO: 30 - protein, 7 aa, Artificial sequence
  FMC63 light chain variable region CDR3 amino acid sequence
QQGNTLP

SEQ ID NO: 31 - protein, 10 aa, Artificial sequence
  M971 heavy chain variable region CDR1 amino acid sequence
GDSVSSNSAA

SEQ ID NO: 32 - protein, 9 aa, Artificial sequence
  M971 heavy chain variable region CDR2 amino acid sequence
TYYRSKWYN

SEQ ID NO: 33 - protein, 2 aa, Artificial sequence
  M971 heavy chain variable region CDR3 amino acid sequence
AR

SEQ ID NO: 34 - protein, 6 aa, Artificial sequence
  M971 light chain variable region CDR1 amino acid sequence
QTIWSY

SEQ ID NO: 35 - protein, 3 aa, Artificial sequence
  M971 light chain variable region CDR2 amino acid sequence
AAS

SEQ ID NO: 36 - protein, 7 aa, Artificial sequence
  M971 light chain variable region CDR3 amino acid sequence
QQSYSIP

SEQ ID NO: 37 - protein, 375 aa, Artificial sequence
  CD19-22 STAR(NCT) alpha chain
DIQMTQTTSSLSASLGDRVTISCRASQDISKYLNWYQQKPDGTVKLLIYHTSRLHSGVPSRFSGSGSGTDYSLTISNLEQEDIATYFCQQGNTLPYTFGGGTKLEITGGGGSGGGGSGGGGSEVKLQESGPGLVAPSQSLSVTCTVSGVSLPDYGVSWIRQPPRKGLEWLGVIWGSETTYYNSALKSRLTIIKDNSKSQVFLKMNSLQTDDTAIYYCAKHYYYGGSYAMDYWGQGTSVTVSSDIQNPDPAVYQLRDDSTLCLFTDFDSQINVPKTMESGTFITDKCVLDMKAMDSKSNGAIAWSNQTSFTCQDIFKETNATYPSSDVPCDATLTEKSFETDMNLNFQNLLVIVLRILLLKVAGFNLLMTLRLWSS

SEQ ID NO: 38 - protein, 472 aa, Artificial sequence
  CD19-22 STAR(NCT) beta chain
DIQMTQSPSSLSASVGDRVTITCRASQTIWSYLNWYQQRPGKAPNLLIYAASSLQSGVPSRFSGRGSGTDFTLTISSLQAEDFATYYCQQSYSIPQTFGQGTKLEIKGGGGSGGGGSGGGGSQVQLQQSGPGLVKPSQTLSLTCAISGDSVSSNSAAWNWIRQSPSRGLEWLGRTYYRSKWYNDYAVSVKSRITINPDTSKNQFSLQLNSVTPEDTAVYYCAREVTGDLEDAFDIWGQGTMVTVSSEFSHFVPVFLPAKPTTTPAPRPPTPAPTIASQPLSLRPEACRPAAGGAVHTRGLDFACDEDLKNVFPPEVAVFEPSAEIATLVCLARGFFPDHVELSWWVNGKEVHSGVCTDPQAYKESNYSYCLSSRLRVSATFWHNPRNHFRCQVQFHGLSEEDKWPEGSPKPVTQNISAEAWGRADCGITSASYQQGVLSATILYEILLGKATLYAVLVSTLVVMAMVKRKNS

SEQ ID NO: 39 - protein, 135 aa, Artificial sequence
  Endodomain-deleted mouse T cell receptor alpha chain constant region
DIQNPEPAVYQLKDPRSQDSTLCLFTDFDSQINVPKTMESGTFITDKTVLDMKAMDSKSNGAIAWSNQTSFTCQDIFKETNATYPSSDVPCDATLTEKSFETDMNLNFQNLSVMGLRILLLKVAGFNLLMTLRLW

SEQ ID NO: 40 - protein, 135 aa, Artificial sequence
  Endodomain-deleted mouse T cell receptor alpha chain constant region with cysteine substitution and hydrophobic modification
DIQNPEPAVYQLKDPRSQDSTLCLFTDFDSQINVPKTMESGTFITDKCVLDMKAMDSKSNGAIAWSNQTSFTCQDIFKETNATYPSSDVPCDATLTEKSFETDMNLNFQNLLVIVLRILLLKVAGFNLLMTLRLW

SEQ ID NO: 41 - protein, 131 aa, Artificial sequence
  Endodomain-deleted mouse T cell receptor alpha chain constant region with N-terminal modification, cysteine substitution and modification of transmembrane hydrophobic region
DIQNPDPAVYQLRDDSTLCLFTDFDSQINVPKTMESGTFITDKCVLDMKAMDSKSNGAIAWSNQTSFTCQDIFKETNATYPSSDVPCDATLTEKSFETDMNLNFQNLLVIVLRILLLKVAGFNLLMTLRLW

SEQ ID NO: 42 - protein, 166 aa, Artificial sequence
  Endodomain-deleted mouse T cell receptor beta chain constant region
DLRNVTPPKVSLFEPSKAEIANKQKATLVCLARGFFPDHVELSWWVNGKEVHSGVSTDPQAYKESNYSYCLSSRLRVSATFWHNPRNHFRCQVQFHGLSEEDKWPEGSPKPVTQNISAEAWGRADCGITSASYQQGVLSATILYEILLGKATLYAVLVSTLVVMAM

SEQ ID NO: 43 - protein, 166 aa, Artificial sequence
  Endodomain-deleted mouse T cell receptor beta chain constant region with cysteine substitution
DLRNVTPPKVSLFEPSKAEIANKQKATLVCLARGFFPDHVELSWWVNGKEVHSGVCTDPQAYKESNYSYCLSSRLRVSATFWHNPRNHFRCQVQFHGLSEEDKWPEGSPKPVTQNISAEAWGRADCGITSASYQQGVLSATILYEILLGKATLYAVLVSTLVVMAM

SEQ ID NO: 44 - protein, 160 aa, Artificial sequence
  Endodomain-deleted mouse T cell receptor beta chain constant region with N-terminal modification and cysteine substitution
DLKNVFPPEVAVFEPSAEIATLVCLARGFFPDHVELSWWVNGKEVHSGVCTDPQAYKESNYSYCLSSRLRVSATFWHNPRNHFRCQVQFHGLSEEDKWPEGSPKPVTQNISAEAWGRADCGITSASYQQGVLSATILYEILLGKATLYAVLVSTLVVMAM

SEQ ID NO: 45 - protein, 108 aa, Artificial sequence
  Anti-CD22 HA22 VL
DIQMTQTTSSLSASLGDRVTISCRASQDISNYLNWYQQKPDGTVKLLIYYTSILHSGVPSRFSGSGSGTDYSLTISNLEQEDFATYFCQQGNTLPWTFGGGTKLEIKA

SEQ ID NO: 46 - protein, 122 aa, Artificial sequence
  Anti-CD22 HA22 VH
EVQLVESGGGLVKPGGSLKLSCAASGFAFSIYDMSWVRQTPEKRLEWVAYISSGGGTYYPDTVKGRFTISRDNAKNTLYLQMSSLKSEDTAMYYCARHSGYGSSYGVLFAYWGQGTLVTVSA

SEQ ID NO: 47 - protein, 418 aa, Artificial sequence
  HA22-FMC63 dual-target STAR beta chain
DIQMTQTTSSLSASLGDRVTISCRASQDISNYLNWYQQKPDGTVKLLIYYTSILHSGVPSRFSGSGSGTDYSLTISNLEQEDFATYFCQQGNTLPWTFGGGTKLEIKAGGGGSGGGGSGGGGSEVQLVESGGGLVKPGGSLKLSCAASGFAFSIYDMSWVRQTPEKRLEWVAYISSGGGTYYPDTVKGRFTISRDNAKNTLYLQMSSLKSEDTAMYYCARHSGYGSSYGVLFAYWGQGTLVTVSAEDLRNVTPPKVSLFEPSKAEIANKQKATLVCLARGFFPDHVELSWWVNGKEVHSGVCTDPQAYKESNYSYCLSSRLRVSATFWHNPRNHFRCQVQFHGLSEEDKWPEGSPKPVTQNISAEAWGRADCGITSASYQQGVLSATILYEILLGKATLYAVLVSTLVVMAMVKRKNS

SEQ ID NO: 48 - protein, 429 aa, Artificial sequence; identical to SEQ ID NO: 18
  HA22-FMC63 dual-target STAR alpha chain

SEQ ID NO: 49 - protein, 421 aa, Artificial sequence
  HA22(M218)-FMC63 dual-target STAR beta chain
DIQMTQTTSSLSASLGDRVTISCRASQDISNYLNWYQQKPDGTVKLLIYYTSILHSGVPSRFSGSGSGTDYSLTISNLEQEDFATYFCQQGNTLPWTFGGGTKLEIKAGSTSGSGKPGSGEGSTKGEVQLVESGGGLVKPGGSLKLSCAASGFAFSIYDMSWVRQTPEKRLEWVAYISSGGGTYYPDTVKGRFTISRDNAKNTLYLQMSSLKSEDTAMYYCARHSGYGSSYGVLFAYWGQGTLVTVSAEDLRNVTPPKVSLFEPSKAEIANKQKATLVCLARGFFPDHVELSWWVNGKEVHSGVCTDPQAYKESNYSYCLSSRLRVSATFWHNPRNHFRCQVQFHGLSEEDKWPEGSPKPVTQNISAEAWGRADCGITSASYQQGVLSATILYEILLGKATLYAVLVSTLVVMAMVKRKNS

SEQ ID NO: 50 - protein, 429 aa, Artificial sequence; identical to SEQ ID NO: 18
  HA22(M218)-FMC63 dual-target STAR alpha chain

SEQ ID NO: 51 - protein, 423 aa, Artificial sequence
  HA22(4G4S)-FMC63 dual-target STAR beta chain
DIQMTQTTSSLSASLGDRVTISCRASQDISNYLNWYQQKPDGTVKLLIYYTSILHSGVPSRFSGSGSGTDYSLTISNLEQEDFATYFCQQGNTLPWTFGGGTKLEIKAGGGGSGGGGSGGGGSGGGGSEVQLVESGGGLVKPGGSLKLSCAASGFAFSIYDMSWVRQTPEKRLEWVAYISSGGGTYYPDTVKGRFTISRDNAKNTLYLQMSSLKSEDTAMYYCARHSGYGSSYGVLFAYWGQGTLVTVSAEDLRNVTPPKVSLFEPSKAEIANKQKATLVCLARGFFPDHVELSWWVNGKEVHSGVCTDPQAYKESNYSYCLSSRLRVSATFWHNPRNHFRCQVQFHGLSEEDKWPEGSPKPVTQNISAEAWGRADCGITSASYQQGVLSATILYEILLGKATLYAVLVSTLVVMAMVKRKNS

SEQ ID NO: 52 - protein, 429 aa, Artificial sequence; identical to SEQ ID NO: 18
  HA22(4G4S)-FMC63 dual-target STAR alpha chain

SEQ ID NO: 53 - protein, 477 aa, Artificial sequence
  HA22(CD8h)-FMC63 dual-target STAR beta chain
DIQMTQTTSSLSASLGDRVTISCRASQDISNYLNWYQQKPDGTVKLLIYYTSILHSGVPSRFSGSGSGTDYSLTISNLEQEDFATYFCQQGNTLPWTFGGGTKLEIKAGGGGSGGGGSGGGGSEVQLVESGGGLVKPGGSLKLSCAASGFAFSIYDMSWVRQTPEKRLEWVAYISSGGGTYYPDTVKGRFTISRDNAKNTLYLQMSSLKSEDTAMYYCARHSGYGSSYGVLFAYWGQGTLVTVSAEFSHFVPVFLPAKPTTTPAPRPPTPAPTIASQPLSLRPEACRPAAGGAVHTRGLDFACDEDLRNVTPPKVSLFEPSKAEIANKQKATLVCLARGFFPDHVELSWWVNGKEVHSGVCTDPQAYKESNYSYCLSSRLRVSATFWHNPRNHFRCQVQFHGLSEEDKWPEGSPKPVTQNISAEAWGRADCGITSASYQQGVLSATILYEILLGKATLYAVLVSTLVVMAMVKRKNS

SEQ ID NO: 54 - protein, 429 aa, Artificial sequence; identical to SEQ ID NO: 18
  HA22(CD8h)-FMC63 dual-target STAR alpha chain

SEQ ID NO: 55 - protein, 6 aa, Artificial sequence
  HA22VL-CDR1
QDISNY

SEQ ID NO: 56 - protein, 3 aa, Artificial sequence
  HA22VL-CDR2
YTS

SEQ ID NO: 57 - protein, 7 aa, Artificial sequence
  HA22VL-CDR3
QQGNTLP

SEQ ID NO: 58 - protein, 8 aa, Artificial sequence
  HA22VH-CDR1
GFAFSIYD

SEQ ID NO: 59 - protein, 7 aa, Artificial sequence
  HA22VH-CDR2
ISSGGGT

SEQ ID NO: 60 - protein, 2 aa, Artificial sequence
  HA22VH-CDR3
AR

SEQ ID NO: 61 - protein, 6 aa, Artificial sequence
  BL22VL-CDR1
QDISNY

SEQ ID NO: 62 - protein, 3 aa, Artificial sequence
  BL22VL-CDR2
YTS

SEQ ID NO: 63 - protein, 7 aa, Artificial sequence
  BL22VL-CDR3
QQGNTLP

SEQ ID NO: 64 - protein, 108 aa, Artificial sequence; identical to SEQ ID NO: 45
  BL22VL

SEQ ID NO: 65 - protein, 8 aa, Artificial sequence
  BL22VH-CDR1
GFAFSIYD

SEQ ID NO: 66 - protein, 7 aa, Artificial sequence
  BL22VH-CDR2
ISSGGGT

SEQ ID NO: 67 - protein, 2 aa, Artificial sequence
  BL22VH-CDR3
AR

SEQ ID NO: 68 - protein, 122 aa, Artificial sequence
  BL22VH
EVQLVESGGGLVKPGGSLKLSCAASGFAFSIYDMSWVRQTPEKRLEWVAYISSGGGTYYPDTVKGRFTISRDNAKNTLYLQMSSLKSEDTAMYYCARHSGYGTHWGVLFAYWGQGTLVTVSA

SEQ ID NO: 69 - protein, 6 aa, Artificial sequence
  M972VL-CDR1
QSFSNM

SEQ ID NO: 70 - protein, 3 aa, Artificial sequence
  M972VL-CDR2
GVS

SEQ ID NO: 71 - protein, 7 aa, Artificial sequence
  M972VL-CDR3
QQYGDWP

SEQ ID NO: 72 - protein, 108 aa, Artificial sequence
  M972VL
RIVMTQSPGTLSVSPGETATLSCRASQSFSNMLAWYQQKSGQPPRLLIYGVSTRAAGVPARFSGSGSGTEFTLTISNLQSEDFAVYYCQQYGDWPRYTFGQGTKVERK

SEQ ID NO: 73 - protein, 8 aa, Artificial sequence
  M972VH-CDR1
GFTFDDYG

SEQ ID NO: 74 - protein, 8 aa, Artificial sequence
  M972VH-CDR2
INWNGGST

SEQ ID NO: 75 - protein, 2 aa, Artificial sequence
  M972VH-CDR3
AR

SEQ ID NO: 76 - protein, 117 aa, Artificial sequence
  M972VH
VQLVQSGGGVVRPGGSLRLPCAASGFTFDDYGMSWVRQAPGKGLEWVSGINWNGGSTGYADSVKGRFTISRDNAKNSLYLQMNSLRAEDTALYHCARGGDYDAFDIWGQGTMVTVSS

SEQ ID NO: 77 - protein, 6 aa, Artificial sequence
  HRFB4VL-CDR1
QDISNY

SEQ ID NO: 78 - protein, 3 aa, Artificial sequence
  HRFB4VL-CDR2
YTS

SEQ ID NO: 79 - protein, 7 aa, Artificial sequence
  HRFB4VL-CDR3
QQGNTLP

SEQ ID NO: 80 - protein, 108 aa, Artificial sequence
  HRFB4VL
DIQLTQSPSSLSASVGDRVTISCRASQDISNYLNWYQQKPGKAPKLLIYYTSILHSGVPSRFSGSGSGTDYTFTISSLQPEDIATYYCQQGNTLPWTFGGGTKVQIKR

SEQ ID NO: 81 - protein, 8 aa, Artificial sequence
  HRFB4VH-CDR1
GFTFSIYD

SEQ ID NO: 82 - protein, 8 aa, Artificial sequence
  HRFB4VH-CDR2
ISSGGGTT

SEQ ID NO: 83 - protein, 2 aa, Artificial sequence
  HRFB4VH-CDR3
AR

SEQ ID NO: 84 - protein, 123 aa, Artificial sequence
  HRFB4VH
QVQLVQSGAEVKKPGSSVKVSCKASGFTFSIYDMSWVRQAPGQGLEWVAYISSGGGTTYYPDTVKGRFTITADESTNTAYMELSSLRSEDTAFYFCARHSGYGSSYGVLFAYWGQGTLVTVSS